European Patent Application EP 4 644 426 A1, published November 5, 2025. Title: 抗凝血因子XI和/或其活化形式因子XIa的抗体及其用途. Applicant: 甘李药业股份有限公司. The sequence listing filed with the application follows.

SEQUENCE LISTING (86 sequences)

SEQ ID NO: 1 - protein, 614 aa, synthetic construct
ECVTQLLKDTCFEGGDITTVFTPSAKYCQVVCTYHPRCLLFTFTAESPSEDPTRWFTCVLKDSVTETLPRVNRTAAISGYSFKQCSHQISACNKDIYVDLDMKGINYNSSVAKSAQECQERCTDDVHCHFFTYATRQFPSLEHRNICLLKHTQTGTPTRITKLDKVVSGFSLKSCALSNLACIRDIFPNTVFADSNIDSVMAPDAFVCGRICTHHPGCLFFTFFSQEWPKESQRNLCLLKTSESGLPSTRIKKSKALSGFSLQSCRHSIPVFCHSSFYHDTDFLGEELDIVAAKSHEACQKLCTNAVRCQFFTYTPAQASCNEGKGKCYLKLSSNGSPTKILHGRGGISGYTLRLCKMDNECTTKIKPRIVGGTASVRGEWPWQVTLHTTSPTQRHLCGGSIIGNQWILTAAHCFYGVESPKILRVYSGILNQSEIKEDTSFFGVQEIIIHDQYKMAESGYDIALLKLETTVNYTDSQRPICLPSKGDRNVIYTDCWVTGWGYRKLRDKIQNTLQKAKIPLVTNEECQKRYRGHKITHKMICAGYREGGKDACKGDSGGPLSCKHNEVWHLVGITSWGEGCAQRERPGVYTNVVEYVDWILEKTQAVGGGSGGG

SEQ ID NO: 2 - protein, 658 aa, synthetic construct
MYRMQLLSCIALSLALVTNSECVTQLLKDTCFEGGDITTVFTPSAKYCQVVCTYHPRCLLFTFTAESPSEDPTRWFTCVLKDSVTETLPRVNRTAAISGYSFKQCSHQISACNKDIYVDLDMKGINYNSSVAKSAQECQERCTDDVHCHFFTYATRQFPSLEHRNICLLKHTQTGTPTRITKLDKVVSGFSLKSCALSNLACIRDIFPNTVFADSNIDSVMAPDAFVCGRICTHHPGCLFFTFFSQEWPKESQRNLCLLKTSESGLPSTRIKKSKALSGFSLQSCRHSIPVFCHSSFYHDTDFLGEELDIVAAKSHEACQKLCTNAVRCQFFTYTPAQASCNEGKGKCYLKLSSNGSPTKILHGRGGISGYTLRLCKMDNECTTKIKPRIVGGTASVRGEWPWQVTLHTTSPTQRHLCGGSIIGNQWILTAAHCFYGVESPKILRVYSGILNQSEIKEDTSFFGVQEIIIHDQYKMAESGYDIALLKLETTVNYTDSQRPICLPSKGDRNVIYTDCWVTGWGYRKLRDKIQNTLQKAKIPLVTNEECQKRYRGHKITHKMICAGYREGGKDACKGDSGGPLSCKHNEVWHLVGITSWGEGCAQRERPGVYTNVVEYVDWILEKTQAVGGGSGGGLNDIFEAQKIEWHEGGPPHHHHHH

SEQ ID NO: 3 - protein, 5 aa, synthetic construct
SYGMS

SEQ ID NO: 4 - protein, 17 aa, synthetic construct
TISSGGSFTYYPDSVKG

SEQ ID NO: 5 - protein, 10 aa, synthetic construct
LTSEGYAMEY

SEQ ID NO: 6 - protein, 15 aa, synthetic construct
RASKSVSTSGYSHMH

SEQ ID NO: 7 - protein, 7 aa, synthetic construct
LASNLES

SEQ ID NO: 8 - protein, 9 aa, synthetic construct
QHSRELPYT

SEQ ID NO: 9 - protein, 5 aa, synthetic construct
NYLIE

SEQ ID NO: 10 - protein, 17 aa, synthetic construct
VINPGSGYTNYNENFKD

SEQ ID NO: 11 - protein, 11 aa, synthetic construct
TYGKYGGAMDF

SEQ ID NO: 12 - protein, 11 aa, synthetic construct
KASQSVSNDVA

SEQ ID NO: 13 - protein, 7 aa, synthetic construct
YISNRYT

SEQ ID NO: 14 - protein, 9 aa, synthetic construct
QQDYSSPPT

SEQ ID NO: 15 - protein, 6 aa, synthetic construct
SGFYWN

SEQ ID NO: 16 - protein, 16 aa, synthetic construct
YISFDGRHNYNPSLKN

SEQ ID NO: 17 - protein, 13 aa, synthetic construct
DLITTVYYYPMDY

SEQ ID NO: 18 - protein, 11 aa, synthetic construct
KASQDVGTAVD

SEQ ID NO: 19 - protein, 7 aa, synthetic construct
WASTRHT

SEQ ID NO: 20 - protein, 9 aa, synthetic construct
QQYSNYPLT

SEQ ID NO: 21 - protein, 5 aa, synthetic construct
DYFIE

SEQ ID NO: 22 - protein, 17 aa, synthetic construct
VINPGNDVTNYNEKFKG

SEQ ID NO: 23 - protein, 11 aa, synthetic construct
SAGNYENSMDF

SEQ ID NO: 24 - protein, 11 aa, synthetic construct
KASQSVSNDVG

SEQ ID NO: 25 - protein, 7 aa, synthetic construct
YTSNRYT

SEQ ID NO: 26 - protein, 9 aa, synthetic construct
QQDYHFPLT

SEQ ID NO: 27 - protein, 5 aa, synthetic construct
NYGVN

SEQ ID NO: 28 - protein, 17 aa, synthetic construct
WINTYTGEPIYADDFKG

SEQ ID NO: 29 - protein, 15 aa, synthetic construct
LYLYGNTYDYYAMDY

SEQ ID NO: 30 - protein, 11 aa, synthetic construct
KASQDISTYLS

SEQ ID NO: 31 - protein, 7 aa, synthetic construct
RANRLID

SEQ ID NO: 32 - protein, 8 aa, synthetic construct
LQYDDLNT

SEQ ID NO: 33 - protein, 5 aa, synthetic construct
DTYMH

SEQ ID NO: 34 - protein, 17 aa, synthetic construct
RIDPANDNTKYDPKFQG

SEQ ID NO: 35 - protein, 9 aa, synthetic construct
DYDGYAMDY

SEQ ID NO: 36 - protein, 11 aa, synthetic construct
KASQDINKYVA

SEQ ID NO: 37 - protein, 7 aa, synthetic construct
YTSTLEP

SEQ ID NO: 38 - protein, 8 aa, synthetic construct
LQYDNLLT

SEQ ID NO: 39 - protein, 5 aa, synthetic construct
GYFMN

SEQ ID NO: 40 - protein, 17 aa, synthetic construct
FINCYNGATSYNQKFKG

SEQ ID NO: 41 - protein, 10 aa, synthetic construct
TISTGDSFDY

SEQ ID NO: 42 - protein, 11 aa, synthetic construct
KASDHINNWLA

SEQ ID NO: 43 - protein, 7 aa, synthetic construct
GASRLET

SEQ ID NO: 44 - protein, 9 aa, synthetic construct
QQYWTTPFT

SEQ ID NO: 45 - protein, 5 aa, synthetic construct
NYLID

SEQ ID NO: 46 - protein, 17 aa, synthetic construct
VINPGSGITNYNEKFKG

SEQ ID NO: 47 - protein, 12 aa, synthetic construct
GDGTYYEDFLDY

SEQ ID NO: 48 - protein, 11 aa, synthetic construct
KASQDINSYLS

SEQ ID NO: 49 - protein, 7 aa, synthetic construct
RANRLMD

SEQ ID NO: 50 - protein, 9 aa, synthetic construct
LQYDEFPLT

SEQ ID NO: 51 - protein, 119 aa, synthetic construct
EVQLQESGGDLVKPGGSLKLSCAASGFTFSSYGMSWVRQTPDKRLEWVATISSGGSFTYYPDSVKGRFTISRDNAKNTLYLQMSSLKSEDTAMYYCASLTSEGYAMEYWGQGTSVTVSS

SEQ ID NO: 52 - protein, 111 aa, synthetic construct
DIVLTQSPASLAVSLGQRATISCRASKSVSTSGYSHMHWYQQKLGQPPKLLIYLASNLESGVPARFSGSGSGTDFTLNIHPVEEEDAATYYCQHSRELPYTFGGGTKLEIK

SEQ ID NO: 53 - protein, 120 aa, synthetic construct
QVQLQQSGAELVRPGTSVTVSCKASGYAFSNYLIEWVNQRPGQGLEWIGVINPGSGYTNYNENFKDKATLTADTSSSTAYMQLSSLTSDDSAVYFCARTYGKYGGAMDFWGQGTSVTVSS

SEQ ID NO: 54 - protein, 107 aa, synthetic construct
DIVMTQTPKFLLVSAGDRVTITCKASQSVSNDVAWYQQKPGQSPKLLIYYISNRYTGVPDRFTGSGYGTDFTFTINTVQAEDLAVYFCQQDYSSPPTFGGGTKLEIK

SEQ ID NO: 55 - protein, 122 aa, synthetic construct
EVQLEESGPGLVKPSQSLSLTCSVTGYSITSGFYWNWIRQFPGNKLEWMGYISFDGRHNYNPSLKNRFSITRDTSKNQFFLKLTSVTAEDTATYYCARDLITTVYYYPMDYWGQGTSVTVSS

SEQ ID NO: 56 - protein, 107 aa, synthetic construct
DIVMTQSHKFMSTSVGDRVSITCKASQDVGTAVDWYQQKTGQSPKLLIYWASTRHTGVPDRFTGSGSGTDFTLTISNVQSEDLADYFCQQYSNYPLTFGAGTKLELK

SEQ ID NO: 57 - protein, 120 aa, synthetic construct
QVKLEESGAELVRPGTSVKVSCKASGYAFTDYFIEWIKQRPGQGLEWIGVINPGNDVTNYNEKFKGKATLTVDKSSTTAYMQLSSLTSDDSAVYFCTRSAGNYENSMDFWGQGTSVTVSS

SEQ ID NO: 58 - protein, 107 aa, synthetic construct
DIVLTQSPKFLLVSAGDRVTITCKASQSVSNDVGWYQQKPGQSPKLLIYYTSNRYTGVPDRFTGSGYGTDFTFTISSVQAEDLAVYFCQQDYHFPLTFGAGTKLELK

SEQ ID NO: 59 - protein, 124 aa, synthetic construct
QVKLQESGPELRKPGETVYISCKASGYTFTNYGVNWVKQAPGKGLKWMGWINTYTGEPIYADDFKGRFAFSLETSANTAYLQISNLTNEDTATYFCARLYLYGNTYDYYAMDYWGQGTSVTVSS

SEQ ID NO: 60 - protein, 106 aa, synthetic construct
DIVLTQTPSSMYASLGERVTITCKASQDISTYLSWFQQKPGKSPKTLIYRANRLIDGVPSRFSGSGSGQDFSLTISSLEYEDMGVYYCLQYDDLNTFGGGTKLEIK

SEQ ID NO: 61 - protein, 118 aa, synthetic construct
EVKLEESGAELVKTGASVKLSCTASGFNIKDTYMHWVKQRPEQGLEWIGRIDPANDNTKYDPKFQGRATVTADTSSNTAYLQLISLTSEDTAVYYCAGDYDGYAMDYWGQGTSVTVSS

SEQ ID NO: 62 - protein, 106 aa, synthetic construct
DIVMTQTTSSLSVSLGGKVTITCKASQDINKYVAWFQHKPGKGPRLLMHYTSTLEPGIPSRFSGSGSGRDYSFTISNLEPEDIATYYCLQYDNLLTFGGGTKLEIK

SEQ ID NO: 63 - protein, 119 aa, synthetic construct
EVKLQESGPELVKTGASVKISCKASGYSFTGYFMNWVKQSHGKSLEWIGFINCYNGATSYNQKFKGKATFTVDASSSSAYMQFNSLTSEDSAVYYCARTISTGDSFDYWGQGSTLTVSS

SEQ ID NO: 64 - protein, 107 aa, synthetic construct
DIVMTQSTSYLSVSLGGRVTITCKASDHINNWLAWYQQKPGDAPSLLISGASRLETGVPSRFSGSGSGKDYTLSITSLQTEDVATYYCQQYWTTPFTFGSGTKLEIK

SEQ ID NO: 65 - protein, 121 aa, synthetic construct
EVQLEESGADLVRPGTSVKVSCKASGYAFTNYLIDWLKQRPGQGLEWIGVINPGSGITNYNEKFKGKATLTTDTSSSTAYMQLTNLTSDDSAVYFCARGDGTYYEDFLDYWGQGTSVTVSS

SEQ ID NO: 66 - protein, 107 aa, synthetic construct
DIVLTQTTSSIYTSLGERVTITCKASQDINSYLSWFQQRPGRSPKTLIYRANRLMDGVPSRFSGSGSGRDFSLTISSLDYEDMGIYYCLQYDEFPLTFGAGTKLELK

SEQ ID NO: 67 - protein, 120 aa, synthetic construct
QVQLVQSGAEVKKPGASVKVSCKASGYTFTNYLIEWVRQAPGQGLEWMGVINPGSGYTNYNENFKDRVTMTRDTSISTAYMELSRLRSDDTAVYYCARTYGKYGGAMDFWGQGTTVTVSS

SEQ ID NO: 68 - protein, 107 aa, synthetic construct
DIVMTQSPDSLAVSLGERATINCKASQSVSNDVAWYQQKPGQPPKLLIYYISNRYTGVPDRFSGSGSGTDFTLTISSLQAEDVAVYYCQQDYSSPPTFGGGTKLEIK

SEQ ID NO: 69 - protein, 120 aa, synthetic construct; identical to SEQ ID NO: 67

SEQ ID NO: 70 - protein, 107 aa, synthetic construct
DIVMTQSPDSLAVSLGERATINCKASQSVSNDVAWYQQKPGQPPKLLIYYISNRYTGVPDRFSGSGSGTDFTLTISSLQAEDVAVYFCQQDYSSPPTFGGGTKLEIK

SEQ ID NO: 71 - protein, 120 aa, synthetic construct
QVQLVQSGAEVKKPGASVKVSCKASGYTFTNYLIEWVRQAPGQGLEWIGVINPGSGYTNYNENFKDRATLTADTSISTAYMELSRLRSDDTAVYFCARTYGKYGGAMDFWGQGTTVTVSS

SEQ ID NO: 72 - protein, 107 aa, synthetic construct; identical to SEQ ID NO: 68

SEQ ID NO: 73 - protein, 120 aa, synthetic construct; identical to SEQ ID NO: 71

SEQ ID NO: 74 - protein, 107 aa, synthetic construct; identical to SEQ ID NO: 70

SEQ ID NO: 75 - protein, 120 aa, synthetic construct
QVQLVQSGAEVKKPGASVKVSCKASGYAFSNYLIEWVGQAPGQGLEWMGVINPGSGYTNYNENFKDRVTMTAHTSISTAYMELSRLRSDDTAVYFCARTYGKYGGAMDFWGQGTLVTVSS

SEQ ID NO: 76 - protein, 107 aa, synthetic construct
DIQMTQSPSSLSASVGDRVTITCKASQSVSNDVAWYQQKPGKAPKLLIYYISNRYTGVPSRFSGSGSGTDFTFTISSLQPEDIATYFCQQDYSSPPTFGQGTKLEIK

SEQ ID NO: 77 - protein, 120 aa, synthetic construct
QVQLVQSGAEVKKPGASVKVSCKASGYAFSNYLIEWVGQAPGQGLEWMGVINPGSGYTNYNENFKDRVTMTRHTSISTAYMELSRLRSDDTAVYFCARTYGKYGGAMDFWGQGTLVTVSS

SEQ ID NO: 78 - protein, 107 aa, synthetic construct
DIQMTQSPSSLSASVGDRVTITCKASQSVSNDVAWYQQKPGKAPKLLIYYISNRYTGVPSRFSGSGSGTDFTFTISSLQPEDIATYYCQQDYSSPPTFGQGTKLEIK

SEQ ID NO: 79 - protein, 120 aa, synthetic construct
QVQLVQSGAEVKKPGSSVKVSCKASGYAFSNYLIEWVRQAPGQGLEWMGVINPGSGYTNYNENFKDRVTITADESTSTAYMELSSLRSEDTAVYYCARTYGKYGGAMDFWGQGTTVTVSS

SEQ ID NO: 80 - protein, 107 aa, synthetic construct
DIQMTQSPSFLSASVGDRVTITCKASQSVSNDVAWYQQKPGKAPKLLIYYISNRYTGVPSRFSGSGSGTDFTLTISSLQPEDFATYYCQQDYSSPPTFGQGTKLEIK

SEQ ID NO: 81 - protein, 120 aa, synthetic construct
QVQLVQSGAEVKKPGSSVKVSCKASGYAFSNYLIEWVRQAPGQGLEWMGVINPGSGYTNYNENFKDRVTITADESTSTAYMELSSLRSEDTAVYFCARTYGKYGGAMDFWGQGTTVTVSS

SEQ ID NO: 82 - protein, 107 aa, synthetic construct
DIQMTQSPSFLSASVGDRVTITCKASQSVSNDVAWYQQKPGKAPKLLIYYISNRYTGVPSRFSGSGSGTDFTLTISSLQPEDFATYFCQQDYSSPPTFGQGTKLEIK

SEQ ID NO: 83 - protein, 120 aa, synthetic construct
QVQLVQSGAEVKKPGSSVKVSCKASGGTFSDYFIEWVRQAPGQGLEWMGVINPGNDVTNYNEKFKGRVTITADKSTSTAYMELSSLRSEDTAVYYCARSAGNYENSMDFWGQGTTVTVSS

SEQ ID NO: 84 - protein, 107 aa, synthetic construct
EIVLTQSPATLSLSPGERATLSCKASQSVSNDVGWYQQKPGQAPRLLIYYTSNRYTGIPARFSGSGSGTDFTLTISSLEPEDFAVYYCQQDYHFPLTFGGGTKVEIK

SEQ ID NO: 85 - protein, 330 aa, artificial sequence
ASTKGPSVFPLAPSSKSTSGGTAALGCLVKDYFPEPVTVSWNSGALTSGVHTFPAVLQSSGLYSLSSVVTVPSSSLGTQTYICNVNHKPSNTKVDKRVEPKSCDKTHTCPPCPAPELLGGPSVFLFPPKPKDTLMISRTPEVTCVVVAVSHEDPEVKFNWYVDGVEVHNAKTKPREEQYNSTYRVVSVLTVLHQDWLNGKEYKCKVSNKALAAPIEKTISKAKGQPREPQVYTLPPSREEMTKNQVSLTCLVKGFYPSDIAVEWESNGQPENNYKTTPPVLDSDGSFFLYSKLTVDKSRWQQGNVFSCSVMHEALHNHYTQKSLSLSPGK

SEQ ID NO: 86 - protein, 107 aa, artificial sequence [sequence omitted]